European Patent Specification EP 3 696 547 B1, published August 13, 2025. Title: Peptide derived from GRP78 for Selecting Highly Efficient Stem Cell. Applicant: Seoul National University R&DB Foundation Chungbuk National University Industry-Academic Cooperation Foundation Nano Intelligent Biomedical Engineering Corporation. co. Ltd. The sequence listing filed with the application follows.

SEQUENCE LISTING (20 sequences)

SEQ ID NO: 1 - protein, 32 aa, Artificial Sequence
  GRP78
MEHRTRSWALGLSILGFFALLFSAGFVQQAHA

SEQ ID NO: 2 - protein, 32 aa, Artificial Sequence
  GRP78
MEHRNRSWALGLSILGFFALLFSAGFVQQAHA

SEQ ID NO: 3 - protein, 32 aa, Artificial Sequence
  GRP78
MDHRNRSWALGLSILGFFALLFSAGFVQQAHA

SEQ ID NO: 4 - protein, 14 aa, Artificial Sequence
  GRP78
TFAPEEISAMVLTK

SEQ ID NO: 5 - protein, 12 aa, Artificial Sequence
  GRP78
DAGTIAGLNVMR

SEQ ID NO: 6 - protein, 12 aa, Artificial Sequence
  GRP78
AKFEELNMDLFR

SEQ ID NO: 7 - protein, 23 aa, Artificial Sequence
  GRP78
KPYIQVDIGGGQTKTFAPEEISA

SEQ ID NO: 8 - protein, 20 aa, Artificial Sequence
  GRP78
MVLTKMKETAEAYLGKKVTH

SEQ ID NO: 9 - protein, 17 aa, Artificial Sequence
  GRP78
AVVTVPAYFNDAQRQAT

SEQ ID NO: 10 - protein, 22 aa, Artificial Sequence
  GRP78
KDAGTIAGLNVMRIINEPTAAA

SEQ ID NO: 11 - protein, 22 aa, Artificial Sequence
  GRP78
IAYGLDKREGEKNILVFDLGGG

SEQ ID NO: 12 - protein, 16 aa, Artificial Sequence
  GRP78
TFDVSLLTIDNGVFEV

SEQ ID NO: 13 - protein, 18 aa, Artificial Sequence
  GRP78
VATNGDTHLGGEDFDQRV

SEQ ID NO: 14 - protein, 18 aa, Artificial Sequence
  GRP78
MEHFIKLYKKKTGKDVRK

SEQ ID NO: 15 - protein, 20 aa, Artificial Sequence
  GRP78
CPLTLGIETVGGVMTKLIPR

SEQ ID NO: 16 - protein, 20 aa, Artificial Sequence
  GRP78
NTVVPTKKSQIFSTASDNQP

SEQ ID NO: 17 - protein, 20 aa, Artificial Sequence
  GRP78
TVTIKVYEGERPLTKDNHLL

SEQ ID NO: 18 - protein, 21 aa, Artificial Sequence
  GRP78
GTFDLTGIPPAPRGVPQIEVT

SEQ ID NO: 19 - protein, 654 aa, Artificial Sequence
  Endoplasmic reticulum chaperone BiP
MKLSLVAAMLLLLSAARAEEEDKKEDVGTVVGIDLGTTYSCVGVFKNGRVEIIANDQGNRITPSYVAFTPEGERLIGDAAKNQLTSNPENTVFDAKRLIGRTWNDPSVQQDIKFLPFKVVEKKTKPYIQVDIGGGQTKTFAPEEISAMVLTKMKETAEAYLGKKVTHAVVTVPAYFNDAQRQATKDAGTIAGLNVMRIINEPTAAATAYGLDKREGEKNTLVFDLGGGTFDVSLLTIDNGVFEVVATNGDTHLGGEDFDQRVMEHFIKLYKKKTGKDVRKDNRAVQKLRREVEKAKRALSSQHQARIEIESFYEGEDFSETLTRAKFEELNMDLFRSTMKPVQKVLEDSDLKKSDIDEIVLVGGSTRIPKIQQLVKEFFNGKEPSRGINPDEAVAYGAAVQAGVLSGDQDTGDLVLLDVCPLTLGIETVGGVMTKLIPRNTVVPTKKSQIFSTASDNQPTVTIKVYEGERPLTKDNHLLGTFDLTGIPPAPRGVPQIEVTFEIDVNGILRVTAEDKGTGNKNKITITNDQNRLTPEEIERMVNDAEKFAEEDKKLKERIDTRNELESYAYSLKNQIGDKEKLGGKLSSEDKETMEKAVEEKIEWLESHQDADIEDFKAKKKELEEIVQPIISKLYGSAGPPPTGEEDTAEKDEI

SEQ ID NO: 20 - protein, 8 aa, Artificial Sequence
  GRP78 binding domain
WIFPWIQL